European Patent Application EP 4 170 030 A1, published April 26, 2023. Title: Aptamer against IL-21 and use thereof. Applicant: RIBOMIC INC. The sequence listing filed with the application follows.

SEQUENCE LISTING (53 sequences)

SEQ ID NO: 1 - RNA, 65 nt, Artificial Sequence
  Aptamer binding to human IL-21 selected by SELEX
gggagaagaaccuucaacacgcgacuacucgugauugcccguucugagcccagacgcucugcgcu

SEQ ID NO: 2 - RNA, 65 nt, Artificial Sequence
  Aptamer binding to human IL-21 selected by SELEX
gggagaagaaccuuccacgaccgacuacugucaauggcccguucuuugcccagacgcucugcgcu

SEQ ID NO: 3 - RNA, 51 nt, Artificial Sequence
  Variant from aptamer shown by SEQ ID NO:1
gggagaagaaccuucaacacgcgacuacucgugauugcccguucugagccc

SEQ ID NO: 4 - RNA, 43 nt, Artificial Sequence
  Variant from aptamer shown by SEQ ID NO:1
ggagaaccuucaacacgcgacuacucgugauugcccguucucc

SEQ ID NO: 5 - RNA, 37 nt, Artificial Sequence
  Variant from aptamer shown by SEQ ID NO:1
ggaccuucaacacgcgacuacucgugauugcccgucc

SEQ ID NO: 6 - RNA, 27 nt, Artificial Sequence
  Variant from aptamer shown by SEQ ID NO:1
ggcaacacgcgacuacucgugauugcc

SEQ ID NO: 7 - RNA, 35 nt, Artificial Sequence
  Variant from aptamer shown by SEQ ID NO:5
ggccuucaacacgcgacuacucgugauugcccgcc

SEQ ID NO: 8 - RNA, 35 nt, Artificial Sequence
  Variant from aptamer shown by SEQ ID NO:7
ggacuucaacacgcgacuacucgugauugcccucc

SEQ ID NO: 9 - RNA, 36 nt, Artificial Sequence
  Variant from aptamer shown by SEQ ID NO:5
ggacuucaacacgcgacuacucgugauugcccgucc

SEQ ID NO: 10 - RNA, 36 nt, Artificial Sequence
  Variant from aptamer shown by SEQ ID NO:5
ggaccucaacacgcgacuacucgugauugcccgucc

SEQ ID NO: 11 - RNA, 36 nt, Artificial Sequence
  Variant from aptamer shown by SEQ ID NO:5
ggaccuucaacacggacuacucgugauugcccgucc

SEQ ID NO: 12 - RNA, 36 nt, Artificial Sequence
  Variant from aptamer shown by SEQ ID NO:5
ggaccuucaacacgcacuacucgugauugcccgucc

SEQ ID NO: 13 - RNA, 36 nt, Artificial Sequence
  Variant from aptamer shown by SEQ ID NO:5
ggaccuucaacacgcgcuacucgugauugcccgucc

SEQ ID NO: 14 - RNA, 36 nt, Artificial Sequence
  Variant from aptamer shown by SEQ ID NO:5
ggaccuucaacacgcgauacucgugauugcccgucc

SEQ ID NO: 15 - RNA, 36 nt, Artificial Sequence
  Variant from aptamer shown by SEQ ID NO:5
ggaccuucaacacgcgacacucgugauugcccgucc

SEQ ID NO: 16 - RNA, 36 nt, Artificial Sequence
  Variant from aptamer shown by SEQ ID NO:5
ggaccuucaacacgcgacucucgugauugcccgucc

SEQ ID NO: 17 - RNA, 36 nt, Artificial Sequence
  Variant from aptamer shown by SEQ ID NO:5
ggaccuucaacacgcgacuaucgugauugcccgucc

SEQ ID NO: 18 - RNA, 36 nt, Artificial Sequence
  Variant from aptamer shown by SEQ ID NO:5
ggaccuucaacacgcgacuaccgugauugcccgucc

SEQ ID NO: 19 - RNA, 36 nt, Artificial Sequence
  Variant from aptamer shown by SEQ ID NO:5
ggaccuucaacacgcgacuacucgugauugccgucc

SEQ ID NO: 20 - RNA, 35 nt, Artificial Sequence
  Variant from aptamer shown by SEQ ID NO:5
gaccuucaacacgcgacuacucgugauugcccguc

SEQ ID NO: 21 - RNA, 33 nt, Artificial Sequence
  Variant from aptamer shown by SEQ ID NO:20
accuucaacacgcgacuacucgugauugcccgu

SEQ ID NO: 22 - RNA, 37 nt, Artificial Sequence
  Variant from aptamer shown by SEQ ID NO:5
ggaccuucaacacgcggcuacucgugauugcccgucc

SEQ ID NO: 23 - RNA, 37 nt, Artificial Sequence
  Variant from aptamer shown by SEQ ID NO:5
gaaccuucaacacgcgacuacucgugauugcccguuc

SEQ ID NO: 24 - RNA, 35 nt, Artificial Sequence
  Variant from aptamer shown by SEQ ID NO:22
gaccuucaacacgcggcuacucgugauugcccguc

SEQ ID NO: 25 - RNA, 37 nt, Artificial Sequence
  Aptamer binding to human IL-21 selected by SELEX
ggaccuucaacacgcgauuacucgugauugcccgucc

SEQ ID NO: 26 - RNA, 37 nt, Artificial Sequence
  Aptamer binding to human IL-21 selected by SELEX
ggaccuucaacaagcgauuacucuugauugcacgucc

SEQ ID NO: 27 - RNA, 37 nt, Artificial Sequence
  Aptamer binding to human IL-21 selected by SELEX
ggaccuucaacccgcgauuacucgggauugcccgucc

SEQ ID NO: 28 - RNA, 37 nt, Artificial Sequence
  Aptamer binding to human IL-21 selected by SELEX
ggaccuucaacccgcgacuacucgggauugcccgucc

SEQ ID NO: 29 - RNA, 37 nt, Artificial Sequence
  Aptamer binding to human IL-21 selected by SELEX
ggcccgccaacacacgauuacuugugauuguccggcc

SEQ ID NO: 30 - RNA, 37 nt, Artificial Sequence
  Aptamer binding to human IL-21 selected by SELEX
ggaccuucaacacgcgauuacucgugauugaccgucc

SEQ ID NO: 31 - RNA, 37 nt, Artificial Sequence
  Aptamer binding to human IL-21 selected by SELEX
ggaccuucaacgcgcgacuacucgcgauugcccgucc

SEQ ID NO: 32 - RNA, 37 nt, Artificial Sequence
  Aptamer binding to human IL-21 selected by SELEX
ggaccgccaacacacgauuacuugugauugcccgucc

SEQ ID NO: 33 - RNA, 37 nt, Artificial Sequence
  Aptamer binding to human IL-21 selected by SELEX
ggaccuucaacccgcgauuacucgggauugcacgucc

SEQ ID NO: 34 - RNA, 37 nt, Artificial Sequence
  Aptamer binding to human IL-21 selected by SELEX
ggaccgccaacacacgacuacuugugauuguccgucc

SEQ ID NO: 35 - RNA, 37 nt, Artificial Sequence
  Aptamer binding to human IL-21 selected by SELEX
ggaccuucaucacgcgauuacucgugaaugcccgucc

SEQ ID NO: 36 - RNA, 37 nt, Artificial Sequence
  Aptamer binding to human IL-21 selected by SELEX
ggaccgccaacaaacgauuacuuuugauuguccgucc

SEQ ID NO: 37 - RNA, 37 nt, Artificial Sequence
  Variant from aptamer shown by SEQ ID NO:28
ggaccuucaacccgcggcuacucgggauugcccgucc

SEQ ID NO: 38 - RNA, 35 nt, Artificial Sequence
  Variant from aptamer shown by SEQ ID NO:37
gaccuucaacccgcggcuacucgggauugcccguc

SEQ ID NO: 39 - RNA, 37 nt, Artificial Sequence
  Variant from aptamer shown by SEQ ID NO:5
ggaccgucaacacgcgacuacucgugauugcccgucc

SEQ ID NO: 40 - RNA, 37 nt, Artificial Sequence
  Variant from aptamer shown by SEQ ID NO:5
ggaccuccaacacgcgacuacucgugauugcccgucc

SEQ ID NO: 41 - RNA, 37 nt, Artificial Sequence
  Variant from aptamer shown by SEQ ID NO:5
ggaccuucaacacgcgacgacucgugauugcccgucc

SEQ ID NO: 42 - RNA, 37 nt, Artificial Sequence
  Variant from aptamer shown by SEQ ID NO:5
ggaccuucaacacgcgacuacccgugauugcccgucc

SEQ ID NO: 43 - RNA, 37 nt, Artificial Sequence
  Variant from aptamer shown by SEQ ID NO:5
ggaccuucaacacgcgacuacucgugauugcacgucc

SEQ ID NO: 44 - protein, 162 aa, Homo sapiens
MRSSPGNMERIVICLMVIFLGTLVHKSSSQGQDRHMIRMRQLIDIVDQLKNYVNDLVPEFLPAPEDVETNCEWSAFSCFQKAQLKSANTGNNERIINVSIKKLKRKPPSTNAGRRQKHRLTCPSCDSYEKKPPKEFLERFKSLLQKMIHQHLSSRTHGSEDS

SEQ ID NO: 45 - protein, 538 aa, Homo sapiens
MPRGWAAPLLLLLLQGGWGCPDLVCYTDYLQTVICILEMWNLHPSTLTLTWQDQYEELKDEATSCSLHRSAHNATHATYTCHMDVFHFMADDIFSVNITDQSGNYSQECGSFLLAESIKPAPPFNVTVTFSGQYNISWRSDYEDPAFYMLKGKLQYELQYRNRGDPWAVSPRRKLISVDSRSVSLLPLEFRKDSSYELQVRAGPMPGSSYQGTWSEWSDPVIFQTQSEELKEGWNPHLLLLLLLVIVFIPAFWSLKTHPLWRLWKKIWAVPSPERFFMPLYKGCSGDFKKWVGAPFTGSSLELGPWSPEVPSTLEVYSCHPPRSPAKRLQLTELQEPAELVESDGVPKPSFWPTAQNSGGSAYSEERDRPYGLVSIDTVTVLDAEGPCTWPCSCEDDGYPALDLDAGLEPSPGLEDPLLDAGTTVLSCGCVSAGSPGLGGPLGSLLDRLKPPLADGEDWAGGLPWGGRSPGGVSESEAGSPLAGLDMDTFDSGFVGSDCSSPVECDFTSPGDEGPPRSYLRQWVVIPPPLSSPGPQAS

SEQ ID NO: 46 - DNA, 84 bp, Artificial Sequence
  DNA template
  misc_feature (16)..(50): n is a, c, g, or t
agcgcagagcgtctgnnnnnnnnnnnnnnnnnnnnnnnnnnnnnnnnnnngaaggttcttctccctatagtgagtcgtattagg

SEQ ID NO: 47 - DNA, 34 bp, Artificial Sequence
  Primer
cctaatacgactcactatagggagaagaaccttc

SEQ ID NO: 48 - DNA, 15 bp, Artificial Sequence
  Primer
agcgcagagcgtctg

SEQ ID NO: 49 - RNA, 51 nt, Artificial Sequence
  Non-human IL-21 aptamer
gggaagcuccgucgagcuuuccugcauaagcuguauugcagccagcauuua

SEQ ID NO: 50 - RNA, 72 nt, Artificial Sequence
  Non-human IL-21 aptamer
gggaagcuccgucgagcuuuccugcauaagcuguauugcagccagcauuuauuguacgccugcguagcuccu

SEQ ID NO: 51 - DNA, 68 bp, Artificial Sequence
  DNA template
gcagagctcgtgctcagaacgggcaatcacgagtagtcgcgtgttgaaggttcttctcactgtgagcc

SEQ ID NO: 52 - DNA, 32 bp, Artificial Sequence
  Primer
taatacgactcactatagggctcacagtgaga

SEQ ID NO: 53 - DNA, 15 bp, Artificial Sequence
  Primer
gcagagctcgtgctc